European Patent Application EP 4 209 505 A1, published July 12, 2023. Title: Compositions containing peptides and their uses. Applicant: Kola-Gen Pharma Inc. The sequence listing filed with the application follows.

SEQUENCE LISTING (3 sequences)

SEQ ID NO: 1 - protein, 36 aa, Artificial sequence
  MOD_RES （5）．．（5）: 4Hyp
  MOD_RES （8）．．（8）: 4Hyp
  MOD_RES （11）．．（11）: 4Hyp
  MOD_RES （14）．．（14）: 4Hyp
  MOD_RES （17）．．（17）: 4Hyp
  MOD_RES （23）．．（23）: 4Hyp
  MOD_RES （26）．．（26）: 4Hyp
  MOD_RES （29）．．（29）: 4Hyp
  MOD_RES （32）．．（32）: 4Hyp
CCCPXGPXGPXGPXGPXGPRGPXGPXGPXGPXGCCC

SEQ ID NO: 2 - protein, 34 aa, Artificial sequence
  MOD_RES （4）．．（4）: 4Hyp
  MOD_RES （7）．．（7）: 4Hyp
  MOD_RES （10）．．（10）: 4Hyp
  MOD_RES （13）．．（13）: 4Hyp
  MOD_RES （16）．．（16）: 4Hyp
  MOD_RES （22）．．（22）: 4Hyp
  MOD_RES （25）．．（25）: 4Hyp
  MOD_RES （28）．．（28）: 4Hyp
  MOD_RES （31）．．（31）: 4Hyp
CCPXGPXGPXGPXGPXGPRGPXGPXGPXGPXGCC

SEQ ID NO: 3 - protein, 36 aa, Artifical Sequence
  MOD_RES （5）．．（5）: 4Hyp
  MOD_RES （8）．．（8）: 4Hyp
  MOD_RES （11）．．（11）: 4Hyp
  MOD_RES （14）．．（14）: 4Hyp
  MOD_RES （17）．．（17）: 4Hyp
  MOD_RES （23）．．（23）: 4Hyp
  MOD_RES （26）．．（26）: 4Hyp
  MOD_RES （29）．．（29）: 4Hyp
  MOD_RES （32）．．（32）: 4Hyp
CCCPXGPXGPXGPXGFXGERGPXGPXGPXGPXGCCC